European Patent Application EP 4 218 817 A2, published August 2, 2023. Title: METHODS FOR TREATING METABOLIC DISEASES BY INHIBITING MYOSTATIN ACTIVATION. Applicant: Scholar Rock, Inc. Application EP Not Yet Assigned, filed January 5, 2018. The sequence listing filed with the application follows.

SEQUENCE LISTING (118 sequences)

SEQ ID NO: 1 - protein, 6 aa, synthetic construct
  source 1..6: note = Synthetic Polypeptide
SSYGMH

SEQ ID NO: 2 - protein, 10 aa, synthetic construct
  source 1..10: note = Synthetic Polypeptide
GFTFSSYGMH

SEQ ID NO: 3 - protein, 10 aa, synthetic construct
  source 1..10: note = Synthetic Polypeptide
GFAFSSYGMH

SEQ ID NO: 4 - protein, 17 aa, synthetic construct
  source 1..17: note = Synthetic Polypeptide
VISYDGSNKYYADSVKG

SEQ ID NO: 5 - protein, 7 aa, synthetic construct
  source 1..7: note = Synthetic Polypeptide
ISYDGSN

SEQ ID NO: 6 - protein, 17 aa, synthetic construct
  source 1..17: note = Synthetic Polypeptide
VISYDGSIKYYADSVKG

SEQ ID NO: 7 - protein, 7 aa, synthetic construct
  source 1..7: note = Synthetic Polypeptide
ISYDGSI

SEQ ID NO: 8 - protein, 17 aa, synthetic construct
  source 1..17: note = Synthetic Polypeptide
VISYDGNNKYYADSVKG

SEQ ID NO: 9 - protein, 7 aa, synthetic construct
  source 1..7: note = Synthetic Polypeptide
ISYDGNN

SEQ ID NO: 10 - protein, 17 aa, synthetic construct
  source 1..17: note = Synthetic Polypeptide
DLLVRFLEWSHYYGMDV

SEQ ID NO: 11 - protein, 17 aa, synthetic construct
  source 1..17: note = Synthetic Polypeptide
DLLVRFLEWSHKYGMDV

SEQ ID NO: 12 - protein, 13 aa, synthetic construct
  source 1..13: note = Synthetic Polypeptide
SGSSSNIGSNTVH

SEQ ID NO: 13 - protein, 8 aa, synthetic construct
  source 1..8: note = Synthetic Polypeptide
SSNIGSNT

SEQ ID NO: 14 - protein, 13 aa, synthetic construct
  source 1..13: note = Synthetic Polypeptide
SGSTSNIGSNTVH

SEQ ID NO: 15 - protein, 8 aa, synthetic construct
  source 1..8: note = Synthetic Polypeptide
TSNIGSNT

SEQ ID NO: 16 - protein, 13 aa, synthetic construct
  source 1..13: note = Synthetic Polypeptide
SGSSSNIGGNTVH

SEQ ID NO: 17 - protein, 8 aa, synthetic construct
  source 1..8: note = Synthetic Polypeptide
SSNIGGNT

SEQ ID NO: 18 - protein, 7 aa, synthetic construct
  source 1..7: note = Synthetic Polypeptide
SDNQRPS

SEQ ID NO: 19 - skipped

SEQ ID NO: 20 - protein, 7 aa, synthetic construct
  source 1..7: note = Synthetic Polypeptide
SDDQRPS

SEQ ID NO: 21 - skipped

SEQ ID NO: 22 - protein, 10 aa, synthetic construct
  source 1..10: note = Synthetic Polypeptide
AAWDDSLNGV

SEQ ID NO: 23 - protein, 10 aa, synthetic construct
  source 1..10: note = Synthetic Polypeptide
AAWDESLNGV

SEQ ID NO: 24 - protein, 126 aa, synthetic construct
  source 1..126: note = Synthetic Polypeptide
QIQLVQSGGGVVQPGRSLRLSCAASGFTFSSYGMHWVRQAPGKGLEWVAVISYDGSNKYYADSVKGRFTISRDNSKNTLYLQMNSLRAEDTAVYYCARDLLVRFLEWSHYYGMDVWGQGTTVTVSS

SEQ ID NO: 25 - protein, 126 aa, synthetic construct
  source 1..126: note = Synthetic Polypeptide
QVQLVESGGGVVQPGRSLRLSCAASGFTFSSYGMHWVRQAPGKGLEWVAVISYDGSNKYYADSVKGRFTISRDNSKNTLYLQMNSLRAEDTAVYYCARDLLVRFLEWSHYYGMDVWGQGTTVTVSS

SEQ ID NO: 26 - protein, 126 aa, synthetic construct
  source 1..126: note = Synthetic Polypeptide
QIQLVQSGGGVVQPGRSLRLSCAASGFAFSSYGMHWVRQAPGKGLEWVAVISYDGSIKYYADSVKGRFTISRDNSKNTLYLQMNSLRAEDTAVYYCARDLLVRFLEWSHKYGMDVWGQGTTVTVSS

SEQ ID NO: 27 - protein, 126 aa, synthetic construct
  source 1..126: note = Synthetic Polypeptide
QVQLVESGGGVVQPGRSLRLSCAASGFAFSSYGMHWVRQAPGKGLEWVAVISYDGSIKYYADSVKGRFTISRDNSKNTLYLQMNSLRAEDTAVYYCARDLLVRFLEWSHKYGMDVWGQGTTVTVSS

SEQ ID NO: 28 - protein, 126 aa, synthetic construct
  source 1..126: note = Synthetic Polypeptide
QIQLVQSGGGVVQPGRSLRLSCAASGFAFSSYGMHWVRQAPGKGLEWVAVISYDGNNKYYADSVKGRFTISRDNSKNTLYLQMNSLRAEDTAVYYCARDLLVRFLEWSHKYGMDVWGQGTTVTVSS

SEQ ID NO: 29 - protein, 126 aa, synthetic construct
  source 1..126: note = Synthetic Polypeptide
QVQLVESGGGVVQPGRSLRLSCAASGFAFSSYGMHWVRQAPGKGLEWVAVISYDGNNKYYADSVKGRFTISRDNSKNTLYLQMNSLRAEDTAVYYCARDLLVRFLEWSHKYGMDVWGQGTTVTVSS

SEQ ID NO: 30 - protein, 109 aa, synthetic construct
  source 1..109: note = Synthetic Polypeptide
QPVLTQPPSASGTPGQRVTISCSGSSSNIGSNTVHWYQQLPGTAPKLLIYSDNQRPSGVPDRFSGSKSGTSASLVISGLQSDDEADYYCAAWDDSLNGVFGGGTKLTVL

SEQ ID NO: 31 - protein, 109 aa, synthetic construct
  source 1..109: note = Synthetic Polypeptide
QSVLTQPPSASGTPGQRVTISCSGSSSNIGSNTVHWYQQLPGTAPKLLIYSDNQRPSGVPDRFSGSKSGTSASLAISGLQSEDEADYYCAAWDDSLNGVFGGGTKLTVL

SEQ ID NO: 32 - protein, 109 aa, synthetic construct
  source 1..109: note = Synthetic Polypeptide
QPVLTQPPSASGTPGQRVTISCSGSTSNIGSNTVHWYQQLPGTAPKLLIYSDDQRPSGVPDRFSGSKSGTSASLVISGLQSDDEADYYCAAWDESLNGVFGGGTKLTVL

SEQ ID NO: 33 - protein, 109 aa, synthetic construct
  source 1..109: note = Synthetic Polypeptide
QSVLTQPPSASGTPGQRVTISCSGSTSNIGSNTVHWYQQLPGTAPKLLIYSDDQRPSGVPDRFSGSKSGTSASLAISGLQSEDEADYYCAAWDESLNGVFGGGTKLTVL

SEQ ID NO: 34 - protein, 109 aa, synthetic construct
  source 1..109: note = Synthetic Polypeptide
QPVLTQPPSASGTPGQRVTISCSGSSSNIGGNTVHWYQQLPGTAPKLLIYSDDQRPSGVPDRFSGSKSGTSASLVISGLQSDDEADYYCAAWDESLNGVFGGGTKLTVL

SEQ ID NO: 35 - protein, 109 aa, synthetic construct
  source 1..109: note = Synthetic Polypeptide
QSVLTQPPSASGTPGQRVTISCSGSSSNIGGNTVHWYQQLPGTAPKLLIYSDDQRPSGVPDRFSGSKSGTSASLAISGLQSEDEADYYCAAWDESLNGVFGGGTKLTVL

SEQ ID NO: 36 - protein, 98 aa, synthetic construct
  source 1..98: note = Synthetic Polypeptide
QVQLVESGGGVVQPGRSLRLSCAASGFTFSSYGMHWVRQAPGKGLEWVAVISYDGSNKYYADSVKGRFTISRDNSKNTLYLQMNSLRAEDTAVYYCAR

SEQ ID NO: 37 - protein, 98 aa, synthetic construct
  source 1..98: note = Synthetic Polypeptide
QSVLTQPPSASGTPGQRVTISCSGSSSNIGSNTVNWYQQLPGTAPKLLIYSNNQRPSGVPDRFSGSKSGTSASLAISGLQSEDEADYYCAAWDDSLNG

SEQ ID NO: 38 - DNA, 378 bp, synthetic construct
  source 1..378: mol_type = other DNA; note = Synthetic Polynucleotide
cagatccagctggtgcagtctgggggaggcgtggtccagcctgggaggtccctgagactctcctgtgcagcgtctggattcaccttcagtagctatggcatgcactgggtccgccaggctccaggcaaggggctggagtgggtggcagttatatcatatgatggaagtaataaatactatgcagactccgtgaagggccgattcaccatctccagagacaattccaagaacacgctgtatctgcaaatgaacagcctgagagccgaggacacggctgtgtattactgtgcgagagatctcctggtgcgatttttggagtggtcgcactactacggtatggacgtctggggccaagggaccacggtcaccgtctcctca

SEQ ID NO: 39 - DNA, 378 bp, synthetic construct
  source 1..378: mol_type = other DNA; note = Synthetic Polynucleotide
caggtgcagctggtggagtctgggggaggcgtggtccagcctgggaggtccctgagactctcctgtgcagcgtctggattcaccttcagtagctatggcatgcactgggtccgccaggctccaggcaaggggctggagtgggtggcagttatatcatatgatggaagtaataaatactatgcagactccgtgaagggccgattcaccatctccagagacaattccaagaacacgctgtatctgcaaatgaacagcctgagagccgaggacacggctgtgtattactgtgcgagagatctcctggtgcgatttttggagtggtcgcactactacggtatggacgtctggggccaagggaccacggtcaccgtctcctca

SEQ ID NO: 40 - DNA, 378 bp, synthetic construct
  source 1..378: mol_type = other DNA; note = Synthetic Polynucleotide
cagatccagctggtgcagtctgggggaggcgtggtccagcctgggaggtccctgagactctcctgtgcagcgtctggattcgccttcagtagctatggcatgcactgggtccgccaggctccaggcaaggggctggagtgggtggcagttatatcatatgatggaagtatcaaatactatgcagactccgtgaagggccgattcaccatctccagagacaattccaagaacacgctgtatctgcaaatgaacagcctgagagccgaggacacggctgtgtattactgtgcgagagatctcctggtgcgatttttggagtggtcgcacaagtacggtatggacgtctggggccaagggaccacggtcaccgtctcctca

SEQ ID NO: 41 - DNA, 378 bp, synthetic construct
  source 1..378: mol_type = other DNA; note = Synthetic Polynucleotide
caggtgcagctggtggagtctgggggaggcgtggtccagcctgggaggtccctgagactctcctgtgcagcgtctggattcgccttcagtagctatggcatgcactgggtccgccaggctccaggcaaggggctggagtgggtggcagttatatcatatgatggaagtatcaaatactatgcagactccgtgaagggccgattcaccatctccagagacaattccaagaacacgctgtatctgcaaatgaacagcctgagagccgaggacacggctgtgtattactgtgcgagagatctcctggtgcgatttttggagtggtcgcacaagtacggtatggacgtctggggccaagggaccacggtcaccgtctcctca

SEQ ID NO: 42 - DNA, 378 bp, synthetic construct
  source 1..378: mol_type = other DNA; note = Synthetic Polynucleotide
cagatccagctggtgcagtctgggggaggcgtggtccagcctgggaggtccctgagactctcctgtgcagcgtctggattcgccttcagtagctatggcatgcactgggtccgccaggctccaggcaaggggctggagtgggtggcagttatatcatatgatggaaataataaatactatgcagactccgtgaagggccgattcaccatctccagagacaattccaagaacacgctgtatctgcaaatgaacagcctgagagccgaggacacggctgtgtattactgtgcgagagatctcctggtgcgatttttggagtggtcgcacaagtacggtatggacgtctggggccaagggaccacggtcaccgtctcctca

SEQ ID NO: 43 - DNA, 378 bp, synthetic construct
  source 1..378: mol_type = other DNA; note = Synthetic Polynucleotide
caggtgcagctggtggagtctgggggaggcgtggtccagcctgggaggtccctgagactctcctgtgcagcgtctggattcgccttcagtagctatggcatgcactgggtccgccaggctccaggcaaggggctggagtgggtggcagttatatcatatgatggaaataataaatactatgcagactccgtgaagggccgattcaccatctccagagacaattccaagaacacgctgtatctgcaaatgaacagcctgagagccgaggacacggctgtgtattactgtgcgagagatctcctggtgcgatttttggagtggtcgcacaagtacggtatggacgtctggggccaagggaccacggtcaccgtctcctca

SEQ ID NO: 44 - DNA, 327 bp, synthetic construct
  source 1..327: mol_type = other DNA; note = Synthetic Polynucleotide
cagcctgtgctgactcagccaccctcagcgtctgggacccccgggcagagggtcaccatctcttgttctggaagcagctccaacatcggaagtaatactgtccactggtaccagcaactcccaggaacggcccccaaactcctcatctatagtgataatcagcgcccctcaggggtccctgaccgattctctggctccaagtctggcacctcagcctccctggtcatcagtgggctccagtctgacgatgaggctgattattactgtgcagcatgggatgacagcctgaatggggtgttcggcggagggaccaagctgaccgtccta

SEQ ID NO: 45 - DNA, 327 bp, synthetic construct
  source 1..327: mol_type = other DNA; note = Synthetic Polynucleotide
cagtctgtgctgactcagccaccctcagcgtctgggacccccgggcagagggtcaccatctcttgttctggaagcagctccaacatcggaagtaatactgtccactggtaccagcaactcccaggaacggcccccaaactcctcatctatagtgataatcagcgcccctcaggggtccctgaccgattctctggctccaagtctggcacctcagcctccctggccatcagtgggctccagtctgaggatgaggctgattattactgtgcagcatgggatgacagcctgaatggggtgttcggcggagggaccaagctgaccgtccta

SEQ ID NO: 46 - DNA, 327 bp, synthetic construct
  source 1..327: mol_type = other DNA; note = Synthetic Polynucleotide
cagcctgtgctgactcagccaccctcagcgtctgggacccccgggcagagggtcaccatctcttgttctggaagcacctccaacatcggaagtaatactgtccactggtaccagcaactcccaggaacggcccccaaactcctcatctatagtgatgatcagcgcccctcaggggtccctgaccgattctctggctccaagtctggcacctcagcctccctggtcatcagtgggctccagtctgacgatgaggctgattattactgtgcagcatgggatgagagcctgaatggggtgttcggcggagggaccaagctgaccgtccta

SEQ ID NO: 47 - DNA, 327 bp, synthetic construct
  source 1..327: mol_type = other DNA; note = Synthetic Polynucleotide
cagtctgtgctgactcagccaccctcagcgtctgggacccccgggcagagggtcaccatctcttgttctggaagcacctccaacatcggaagtaatactgtccactggtaccagcaactcccaggaacggcccccaaactcctcatctatagtgatgatcagcgcccctcaggggtccctgaccgattctctggctccaagtctggcacctcagcctccctggccatcagtgggctccagtctgaggatgaggctgattattactgtgcagcatgggatgagagcctgaatggggtgttcggcggagggaccaagctgaccgtccta

SEQ ID NO: 48 - DNA, 327 bp, synthetic construct
  source 1..327: mol_type = other DNA; note = Synthetic Polynucleotide
cagcctgtgctgactcagccaccctcagcgtctgggacccccgggcagagggtcaccatctcttgttctggaagcagctccaacatcggaggaaatactgtccactggtaccagcaactcccaggaacggcccccaaactcctcatctatagtgatgatcagcgcccctcaggggtccctgaccgattctctggctccaagtctggcacctcagcctccctggtcatcagtgggctccagtctgacgatgaggctgattattactgtgcagcatgggatgagagcctgaatggggtgttcggcggagggaccaagctgaccgtccta

SEQ ID NO: 49 - DNA, 327 bp, synthetic construct
  source 1..327: mol_type = other DNA; note = Synthetic Polynucleotide
cagtctgtgctgactcagccaccctcagcgtctgggacccccgggcagagggtcaccatctcttgttctggaagcagctccaacatcggaggaaatactgtccactggtaccagcaactcccaggaacggcccccaaactcctcatctatagtgatgatcagcgcccctcaggggtccctgaccgattctctggctccaagtctggcacctcagcctccctggccatcagtgggctccagtctgaggatgaggctgattattactgtgcagcatgggatgagagcctgaatggggtgttcggcggagggaccaagctgaccgtccta

SEQ ID NO: 50 - protein, 452 aa, synthetic construct
  source 1..452: note = Synthetic Polypeptide
QVQLVESGGGVVQPGRSLRLSCAASGFTFSSYGMHWVRQAPGKGLEWVAVISYDGSNKYYADSVKGRFTISRDNSKNTLYLQMNSLRAEDTAVYYCARDLLVRFLEWSHYYGMDVWGQGTTVTVSSASTKGPSVFPLAPCSRSTSESTAALGCLVKDYFPEPVTVSWNSGALTSGVHTFPAVLQSSGLYSLSSVVTVPSSSLGTKTYTCNVDHKPSNTKVDKRVESKYGPPCPPCPAPEFLGGPSVFLFPPKPKDTLMISRTPEVTCVVVDVSQEDPEVQFNWYVDGVEVHNAKTKPREEQFNSTYRVVSVLTVLHQDWLNGKEYKCKVSNKGLPSSIEKTISKAKGQPREPQVYTLPPSQEEMTKNQVSLTCLVKGFYPSDIAVEWESNGQPENNYKTTPPVLDSDGSFFLYSRLTVDKSRWQEGNVFSCSVMHEALHNHYTQKSLSLSLG

SEQ ID NO: 51 - protein, 215 aa, synthetic construct
  source 1..215: note = Synthetic Polypeptide
QSVLTQPPSASGTPGQRVTISCSGSSSNIGSNTVHWYQQLPGTAPKLLIYSDNQRPSGVPDRFSGSKSGTSASLAISGLQSEDEADYYCAAWDDSLNGVFGGGTKLTVLGQPKAAPSVTLFPPSSEELQANKATLVCLISDFYPGAVTVAWKADSSPVKAGVETTTPSKQSNNKYAASSYLSLTPEQWKSHRSYSCQVTHEGSTVEKTVAPTECS

SEQ ID NO: 52 - protein, 352 aa, Homo sapiens [sequence omitted]

SEQ ID NO: 53 - protein, 352 aa, Rattus rattus
NEDSEREANVEKEGLCNACAWRQNTRYSRIEAIKIQILSKLRLETAPNISKDAIRQLLPRAPPLRELIDQYDVQRDDSSDGSLEDDDYHATTETIITMPTESDFLMQADGKPKCCFFKFSSKIQYNKVVKAQLWIYLRAVKTPTTVFVQILRLIKPMKDGTRYTGIRSLKLDMSPGTGIWQSIDVKTVLQNWLKQPESNLGIEIKALDENGHDLAVTFPGPGEDGLNPFLEVKVTDTPKRSRRDFGLDCDEHSTESRCCRYPLTVDFEAFGWDWIIAPKRYKANYCSGECEFVFLQKYPHTHLVHQANPRGSAGPCCTPTKMSPINMLYFNGKEQIIYGKIPAMVVDRCGCS

SEQ ID NO: 54 - protein, 352 aa, Mus musculus
NEGSEREENVEKEGLCNACAWRQNTRYSRIEAIKIQILSKLRLETAPNISKDAIRQLLPRAPPLRELIDQYDVQRDDSSDGSLEDDDYHATTETIITMPTESDFLMQADGKPKCCFFKFSSKIQYNKVVKAQLWIYLRPVKTPTTVFVQILRLIKPMKDGTRYTGIRSLKLDMSPGTGIWQSIDVKTVLQNWLKQPESNLGIEIKALDENGHDLAVTFPGPGEDGLNPFLEVKVTDTPKRSRRDFGLDCDEHSTESRCCRYPLTVDFEAFGWDWIIAPKRYKANYCSGECEFVFLQKYPHTHLVHQANPRGSAGPCCTPTKMSPINMLYFNGKEQIIYGKIPAMVVDRCGCS

SEQ ID NO: 55 - protein, 277 aa, Macaca fascicularis
NENSEQKENVEKEGLCNACTWRQNTKSSRIEAIKIQILSKLRLETAPNISKDAIRQLLPKAPPLRELIDQYDVQRDDSSDGSLEDDDYHATTETIITMPTESDFLMQVDGKPKCCFFKFSSKIQYNKVVKAQLWIYLRPVETPTTVFVQILRLIKPMKDGTRYTGIRSLKLDMNPGTGIWQSIDVKTVLQNWLKQPESNLGIEIKALDENGHDLAVTFPGPGEDGLNPFLEVKVTDTPKRSRRDFGLDCDEHSTESRCCRYPLTVDFEAFGWDWIIA

SEQ ID NO: 56 - protein, 4 aa, synthetic construct
  source 1..4: note = Synthetic Polypeptide
RSRR

SEQ ID NO: 57 - protein, 4 aa, synthetic construct
  source 1..4: note = Synthetic Polypeptide
RVRR

SEQ ID NO: 58 - protein, 5 aa, synthetic construct
  source 1..5: note = Synthetic Polypeptide
CPPCP

SEQ ID NO: 59 - protein, 17 aa, synthetic construct
  source 1..17: note = Synthetic Polypeptide
HYYGMDVWGQGTTVTVS

SEQ ID NO: 60 - protein, 89 aa, synthetic construct
  source 1..89: note = Synthetic Polypeptide
QSVLTQPPSASGTPGQRVTISCSGSSSNIGSNTVNWYQQLPGTAPKLLIYSNNQRPSGVPDRFSGSKSGTSASLAISGLQSEDEADYYC

SEQ ID NO: 61 - protein, 11 aa, synthetic construct
  source 1..11: note = Synthetic Polypeptide
VFGGGTKLTVL

SEQ ID NO: 62 - protein, 33 aa, synthetic construct
  source 1..33: note = Synthetic Polypeptide
PKAPPLRELIDQYDVQRDDSSDGSLEDDDYHAT

SEQ ID NO: 63 - protein, 34 aa, synthetic construct
  source 1..34: note = Synthetic Polypeptide
GLNPFLEVKVTDTPKRSRRDFGLDCDEHSTESRC

SEQ ID NO: 64 - protein, 80 aa, synthetic construct
  source 1..80: note = Synthetic Polypeptide
VDLNENSEQKENVEKEGLCNACTWRQNTKSSRIEAIKIQILSKLRLETAPNISKDVIRQLLPKAPPLRELIDQYDVQRDD

SEQ ID NO: 65 - protein, 418 aa, synthetic construct
  source 1..418: note = Synthetic Polypeptide
MDMRVPAQLLGLLLLWFSGVLGDYKDDDDKHHHHHHLEVLFQGPAEGPAAAAAAAAAAAAAGVGGERSSRPAPSVAPEPDGCPVCVWRQHSRELRLESIKSQILSKLRLKEAPNISREVVKQLLPKAPPLRELIDQYDVQRDDSSDGSLEDDDYHATTETIITMPTESDFLMQVDGKPKCCFFKFSSKIQYNKVVKAQLWIYLRPVETPTTVFVQILRLIKPMKDGTRYTGIRSLKLDMNPGTGIWQSIDVKTVLQNWLKQPESNLGIEIKALDENGHDLAVTFPGPGEDGLNPFLEVKVTDTPKRSRRNLGLDCDEHSSESRCCRYPLTVDFEAFGWDWIIAPKRYKANYCSGQCEYMFMQKYPHTHLVQQANPRGSAGPCCTPTKMSPINMLYFNDKQQIIYGKIPGMVVDRCGCS

SEQ ID NO: 66 - protein, 19 aa, synthetic construct
  source 1..19: note = Synthetic Polypeptide
ARDLLVRFLEWSHYYGMDV

SEQ ID NO: 67 - protein, 10 aa, synthetic construct
  source 1..10: note = Synthetic Polypeptide
AAWDDSLNGV

SEQ ID NO: 68 - protein, 128 aa, synthetic construct
  source 1..128: note = Synthetic Polypeptide
QIQLVQSGGGVVQPGRSLRLSCAASGFTFSSYGMHWVRQAPGKGLEWVAVISYDGSNKYYADSVKGRFTISRDNSKNTLYLQMNSLRAEDTAVYYCARDLLVRFLEWSHYYGMDVWGQGTTVTVSSGS

SEQ ID NO: 69 - protein, 125 aa, synthetic construct
  source 1..125: note = Synthetic Polypeptide
QPVLTQPPSASGTPGQRVTISCSGSSSNIGSNTVHWYQQLPGTAPKLLIYSDNQRPSGVPDRFSGSKSGTSASLVISGLQSDDEADYYCAAWDDSLNGVFGGGTKLTVLGQPKAAPSVTLFSPSS

SEQ ID NO: 70 - protein, 272 aa, synthetic construct
  source 1..272: note = Synthetic Polypeptide
QIQLVQSGGGVVQPGRSLRLSCAASGFTFSSYGMHWVRQAPGKGLEWVAVISYDGSNKYYADSVKGRFTISRDNSKNTLYLQMNSLRAEDTAVYYCARDLLVRFLEWSHYYGMDVWGQGTTVTVSSGSASAPTLGGGGSGGGGSAAAQPVLTQPPSASGTPGQRVTISCSGSSSNIGSNTVHWYQQLPGTAPKLLIYSDNQRPSGVPDRFSGSKSGTSASLVISGLQSDDEADYYCAAWDDSLNGVFGGGTKLTVLGQPKAAPSVTLFSPSS

SEQ ID NO: 71 - protein, 19 aa, synthetic construct
  source 1..19: note = Synthetic Polypeptide
ARESLIRFLEDPQQGGMDV

SEQ ID NO: 72 - protein, 10 aa, synthetic construct
  source 1..10: note = Synthetic Polypeptide
NSWTRSNNYI

SEQ ID NO: 73 - protein, 128 aa, synthetic construct
  source 1..128: note = Synthetic Polypeptide
QVQLQQSGAEVKKPGASVKVSCKASGYTFTSYYMHWVRQAPGQGLEWMGIINPSGGSTSYAQKFQGRVTMTRDTSTSTVYMELSSLRSEDTAVYYCARESLIRFLEDPQQGGMDVWGQGTTVTVSSGS

SEQ ID NO: 74 - protein, 126 aa, synthetic construct
  source 1..126: note = Synthetic Polypeptide
QSALTQPASVSGSPGQSLTISCTGTSSDIGGYNYVSWYQQHPGKAPKLIIYDVTDRPSGVSGRFSGSKSGNTASLTISGLQTEDEAEYFCNSWTRSNNYIFGGGTKLTVLGQPKAAPSVTLFPPSS

SEQ ID NO: 75 - protein, 273 aa, synthetic construct
  source 1..273: note = Synthetic Polypeptide
QVQLQQSGAEVKKPGASVKVSCKASGYTFTSYYMHWVRQAPGQGLEWMGIINPSGGSTSYAQKFQGRVTMTRDTSTSTVYMELSSLRSEDTAVYYCARESLIRFLEDPQQGGMDVWGQGTTVTVSSGSASAPTLGGGGSGGGGSAAAQSALTQPASVSGSPGQSLTISCTGTSSDIGGYNYVSWYQQHPGKAPKLIIYDVTDRPSGVSGRFSGSKSGNTASLTISGLQTEDEAEYFCNSWTRSNNYIFGGGTKLTVLGQPKAAPSVTLFPPSS

SEQ ID NO: 76 - protein, 15 aa, synthetic construct
  source 1..15: note = Synthetic Polypeptide
ARDRYSSSWGGGFDY

SEQ ID NO: 77 - protein, 10 aa, synthetic construct
  source 1..10: note = Synthetic Polypeptide
QSYDASSLWV

SEQ ID NO: 78 - protein, 124 aa, synthetic construct
  source 1..124: note = Synthetic Polypeptide
EVQLVQSGGGVVQSGRSLRLSCVASGFSFSNYGMHWVRQAPGKGLEWLAFIWYDGSNKWYADSVKGRFTISRDNSKNALYLQMNSLRAEDTAVYYCARDRYSSSWGGGFDYWGQGTVLTVSSGS

SEQ ID NO: 79 - protein, 132 aa, synthetic construct
  source 1..132: note = Synthetic Polypeptide
NFMLTQPHSVSESPGRTVTIPCSGRGGSIASDSVQWYQQRPGSAPTTIIYEDNQRPSGVPDRFSGSVDSSSNSASLTISGLRTEDEADYYCQSYDASSLWVFGGKTKLTVLGQPKAAPSVTLFPPSSKASGA

SEQ ID NO: 80 - protein, 275 aa, synthetic construct
  source 1..275: note = Synthetic Polypeptide
EVQLVQSGGGVVQSGRSLRLSCVASGFSFSNYGMHWVRQAPGKGLEWLAFIWYDGSNKWYADSVKGRFTISRDNSKNALYLQMNSLRAEDTAVYYCARDRYSSSWGGGFDYWGQGTVLTVSSGSASAPTLGGGGSGGGGSAAANFMLTQPHSVSESPGRTVTIPCSGRGGSIASDSVQWYQQRPGSAPTTIIYEDNQRPSGVPDRFSGSVDSSSNSASLTISGLRTEDEADYYCQSYDASSLWVFGGKTKLTVLGQPKAAPSVTLFPPSSKASGA

SEQ ID NO: 81 - protein, 12 aa, synthetic construct
  source 1..12: note = Synthetic Polypeptide
VRDRHSLGDFDY

SEQ ID NO: 82 - protein, 9 aa, synthetic construct
  source 1..9: note = Synthetic Polypeptide
QAWDSTTVV

SEQ ID NO: 83 - protein, 121 aa, synthetic construct
  source 1..121: note = Synthetic Polypeptide
QLQLQQSGGGLVKPGGSLRLSCAASGFTFSSYSMNWVRQAPGKGLEWVSSISSSSSYIYYADSVKGRFTISRDNAKNSLYLQMNSLRAEDTAVYYCVRDRHSLGDFDYWGQGTLVTVSSGS

SEQ ID NO: 84 - protein, 121 aa, synthetic construct
  source 1..121: note = Synthetic Polypeptide
SSELTQPSVSVSPGQTATITCSGDKLGDKYASWYQQKPGQSPVLVIYQDTKRPSGIPARFSGSNSGNTATLTISGTQAMDEAAYYCQAWDSTTVVFGGGTKLTVLGQPKAAPSVTLFPPSS

SEQ ID NO: 85 - protein, 201 aa, synthetic construct
  source 1..201: note = Synthetic Polypeptide
QLQLQQSGGGLVKPGGSLRLSCAASGFTFSSYSMNWVRQAPGKGLEWVSSISSSSSYIYYADSVKGRFTISRDNAKNSLYLQMNSLRAEDTAVYYCVRDRHSLGDFDYWGQGTLVTVSSGSASAPTLGGGGSGGGGSAAASSELTQPPSVSVSPGQTATITCSGDKLGDKYASWYQQKPGQSPVLVIYQDTKRPSGIPARF

SEQ ID NO: 86 - protein, 20 aa, synthetic construct
  source 1..20: note = Synthetic Polypeptide
ANHGLMDDSSGYYLSNAFDI

SEQ ID NO: 87 - protein, 11 aa, synthetic construct
  source 1..11: note = Synthetic Polypeptide
ATWDDSLTGVV

SEQ ID NO: 88 - protein, 129 aa, synthetic construct
  source 1..129: note = Synthetic Polypeptide
QVQLVQSGAEVKKPGSSVKVSCKASGGTFSSYAISWVRQAPGQGLEWMGGIIPIFGTANYAQKFQGRVTITADESTSTAYMELSSLRSEDTAVYYCANHGLMDDSSGYYLSNAFDIWGQGTMVTVSSGS

SEQ ID NO: 89 - protein, 126 aa, synthetic construct
  source 1..126: note = Synthetic Polypeptide
QPVLTQPPSASGTPGQRVTISCSGSSSNIGSNTVEWYQQLPGTAPKLLIHSNNQRPSGVPDRFSGSRSGTSASLAISGLQSEDEADYFCATWDDSLTGVVFGGGTTLTVLGQPKAAPSVTLFPPSS

SEQ ID NO: 90 - protein, 274 aa, synthetic construct
  source 1..274: note = Synthetic Polypeptide
QVQLVQSGAEVKKPGSSVKVSCKASGGTFSSYAISWVRQAPGQGLEWMGGIIPIFGTANYAQKFQGRVTITADESTSTAYMELSSLRSEDTAVYYCANHGLMDDSSGYYLSNAFDIWGQGTMVTVSSGSASAPTLGGGGSGGGGSAAAQPVLTQPPSASGTPGQRVTISCSGSSSNIGSNTVEWYQQLPGTAPKLLIHSNNQRPSGVPDRFSGSRSGTSASLAISGLQSEDEADYFCATWDDSLTGVVFGGGTTLTVLGQPKAAPSVTLFPPSS

SEQ ID NO: 91 - protein, 14 aa, synthetic construct
  source 1..14: note = Synthetic Polypeptide
AKVGTAAAGDAFDI

SEQ ID NO: 92 - protein, 11 aa, synthetic construct
  source 1..11: note = Synthetic Polypeptide
AAWDDSLSGWV

SEQ ID NO: 93 - protein, 123 aa, synthetic construct
  source 1..123: note = Synthetic Polypeptide
QVQLVQSGGGLIQPGGSLRLSCAASGFTVSSYSMNWVRQAPGKGLEWVSYISSSGSTIYYADSVKGRFTISRDNAKNSLYLQMNSLRAEDTALYYCAKVGTAAAGDAFDIWGQGTMVTVSSGS

SEQ ID NO: 94 - protein, 126 aa, synthetic construct
  source 1..126: note = Synthetic Polypeptide
QPVLTQPPSASGTPGQRVTISCFGSSSNIGSNYVYWYQQLPGTAPKLLIYRNNQRPSGVPDRFSGSKSGTSASLAISGLRSEDEADYYCAAWDDSLSGWVFGGGTKLTVLGQPKAAPSVTLFPPSS

SEQ ID NO: 95 - protein, 268 aa, synthetic construct
  source 1..268: note = Synthetic Polypeptide
QVQLVQSGGGLIQPGGSLRLSCAASGFTVSSYSMNWVRQAPGKGLEWVSYISSSGSTIYYADSVKGRFTISRDNAKNSLYLQMNSLRAEDTALYYCAKVGTAAAGDAFDIWGQGTMVTVSSGSASAPTLGGGGSGGGGSAAAQPVLTQPPSASGTPGQRVTISCFGSSSNIGSNYVYWYQQLPGTAPKLLIYRNNQRPSGVPDRFSGSKSGTSASLAISGLRSEDEADYYCAAWDDSLSGWVFGGGTKLTVLGQPKAAPSVTLFPPSS

SEQ ID NO: 96 - protein, 20 aa, synthetic construct
  source 1..20: note = Synthetic Polypeptide
ARVGFYDYVWGSYPYDAFDI

SEQ ID NO: 97 - protein, 9 aa, synthetic construct
  source 1..9: note = Synthetic Polypeptide
QQYGTSPLT

SEQ ID NO: 98 - protein, 129 aa, synthetic construct
  source 1..129: note = Synthetic Polypeptide
QIQLVQSGAEVKKPGASVKVSCKASGYTFTSYGISWVRQAPGQGLEWMGWISAYNGNTNYAQKLQGRVTMTTDTSTSTAYMELSSLRSEDTAVYYCARVGFYDYVWGSYPYDAFDIWGQGTMVTVSSGS

SEQ ID NO: 99 - protein, 117 aa, synthetic construct
  source 1..117: note = Synthetic Polypeptide
EIVMTQSPGTLSLSPGERATLSCRASQSVSSNYLAWYQQKPGQAPRLLIYDASNRATGIPARFSGSGSGTDFTLTISSLEPEDFALYYCQQYGTSPLTFGGGTKLEIKRTVAAPSVF

SEQ ID NO: 100 - protein, 265 aa, synthetic construct
  source 1..265: note = Synthetic Polypeptide
QIQLVQSGAEVKKPGASVKVSCKASGYTFTSYGISWVRQAPGQGLEWMGWISAYNGNTNYAQKLQGRVTMTTDTSTSTAYMELSSLRSEDTAVYYCARVGFYDYVWGSYPYDAFDIWGQGTMVTVSSGSASAPTLGGGGSGGGGSAAAEIVMTQSPGTLSLSPGERATLSCRASQSVSSNYLAWYQQKPGQAPRLLIYDASNRATGIPARFSGSGSGTDFTLTISSLEPEDFALYYCQQYGTSPLTFGGGTKLEIKRTVAAPSVF

SEQ ID NO: 101 - protein, 16 aa, synthetic construct
  source 1..16: note = Synthetic Polypeptide
AKDTSNGGYSSSSFDY

SEQ ID NO: 102 - protein, 10 aa, synthetic construct
  source 1..10: note = Synthetic Polypeptide
SSYTSSSTLV

SEQ ID NO: 103 - protein, 125 aa, synthetic construct
  source 1..125: note = Synthetic Polypeptide
EVQLVQSGGGLVQPGRSLRLSCAASGFTFDDYAMHWVRQAPGKGLEWVSGISWNSGSIGYADSVKGRFTISRDNAKNSLYLQMNSLRAEDTALYYCAKDTSNGGYSSSSFDYWGQGTLVTVSSGS

SEQ ID NO: 104 - protein, 126 aa, synthetic construct
  source 1..126: note = Synthetic Polypeptide
QSALTQPASVSGSPGQSITISCTGTSSDVGGYNYVSWYQQHPGTAPKLMIYDVSYRPSGVSNRFSGSKSGNTASLTISGLQAEDEADYYCSSYTSSSTLVFGTGTKVTVLGQPKANPTVTLFPPSS

SEQ ID NO: 105 - protein, 270 aa, synthetic construct
  source 1..270: note = Synthetic Polypeptide
EVQLVQSGGGLVQPGRSLRLSCAASGFTFDDYAMHWVRQAPGKGLEWVSGISWNSGSIGYADSVKGRFTISRDNAKNSLYLQMNSLRAEDTALYYCAKDTSNGGYSSSSFDYWGQGTLVTVSSGSASAPTLGGGGSGGGGSAAAQSALTQPASVSGSPGQSITISCTGTSSDVGGYNYVSWYQQHPGTAPKLMIYDVSYRPSGVSNRFSGSKSGNTASLTISGLQAEDEADYYCSSYTSSSTLVFGTGTKVTVLGQPKANPTVTLFPPSS

SEQ ID NO: 106 - protein, 17 aa, synthetic construct
  source 1..17: note = Synthetic Polypeptide
ARLVYGGYDEPGYYFDY

SEQ ID NO: 107 - protein, 11 aa, synthetic construct
  source 1..11: note = Synthetic Polypeptide
AAWDDSLNGWV

SEQ ID NO: 108 - protein, 126 aa, synthetic construct
  source 1..126: note = Synthetic Polypeptide
EVQLLESRAEVKKPGESLKISCKGSGYSFTSYWIGWVRQMPGKGPEWMGIIYPGDSDTRYSPSFQGQVTISADKSISTAYLQWSSLKASDTAMYYCARLVYGGYDEPGYYFDYWGQGTLVTVSSGS

SEQ ID NO: 109 - protein, 131 aa, synthetic construct
  source 1..131: note = Synthetic Polypeptide
QSVLTQPPSASGTPGQRVTISCSGSSSNIRSNTVNWYQQLPGTAPKLLIYSNNQRPSGVPDRFSGSKSGTSASLAISGLQSEDEADYYCAAWDDSLNGWVFGGGTKLTVLGQPKAAPSVTLFPPSSKASGA

SEQ ID NO: 110 - protein, 276 aa, synthetic construct
  source 1..276: note = Synthetic Polypeptide
EVQLLESRAEVKKPGESLKISCKGSGYSFTSYWIGWVRQMPGKGPEWMGIIYPGDSDTRYSPSFQGQVTISADKSISTAYLQWSSLKASDTAMYYCARLVYGGYDEPGYYFDYWGQGTLVTVSSGSASAPTLGGGGSGGGGSAAAQSVLTQPPSASGTPGQRVTISCSGSSSNIRSNTVNWYQQLPGTAPKLLIYSNNQRPSGVPDRFSGSKSGTSASLAISGLQSEDEADYYCAAWDDSLNGWVFGGGTKLTVLGQPKAAPSVTLFPPSSKASGA

SEQ ID NO: 111 - protein, 16 aa, synthetic construct
  source 1..16: note = Synthetic Polypeptide
AKVDGLEYSSGHNFDY

SEQ ID NO: 112 - protein, 10 aa, synthetic construct
  source 1..10: note = Synthetic Polypeptide
SSYAGSYTWV

SEQ ID NO: 113 - protein, 125 aa, synthetic construct
  source 1..125: note = Synthetic Polypeptide
EVQLVQSGGGLVQPGRSLRLSCAASGFTFDDYAMHWVRQAPGKGLEWVSGISWNSGSIGYADSVKGRFTISRDNSKNTLYLQMNSLRAEDTAVYYCAKVDGLEYSSGHNFDYWGQGTLVTVSSGS

SEQ ID NO: 114 - protein, 126 aa, synthetic construct
  source 1..126: note = Synthetic Polypeptide
QSALTQPPSVSGSPGQSVTISCTGSSSDVGYYDHVSWYQHHPGRAPKVIIYDVTKRPSGVPDRFSGSKSGNTASLTISGLQAEDEADYYCSSYAGSYTWVFGGGTELTVLGQPKAAPSVTLFPPSS

SEQ ID NO: 115 - protein, 270 aa, synthetic construct
  source 1..270: note = Synthetic Polypeptide
EVQLVQSGGGLVQPGRSLRLSCAASGFTFDDYAMHWVRQAPGKGLEWVSGISWNSGSIGYADSVKGRFTISRDNSKNTLYLQMNSLRAEDTAVYYCAKVDGLEYSSGHNFDYWGQGTLVTVSSGSASAPTLGGGGSGGGGSAAAQSALTQPPSVSGSPGQSVTISCTGSSSDVGYYDHVSWYQHHPGRAPKVIIYDVTKRPSGVPDRFSGSKSGNTASLTISGLQAEDEADYYCSSYAGSYTWVFGGGTELTVLGQPKAAPSVTLFPPSS

SEQ ID NO: 116 - protein, 323 aa, synthetic construct
  source 1..323: note = Synthetic Polypeptide
ASTTPPSVYPLAPGSAAQTNSMVTLGCLVKGYFPEPVTVTWNSGSLSSGVHTFPAVLQSDLYTLSSSVTVPSSTWPSETVTCNVAHPASSTKVDKKIVPRDCGCKPCICTVPEVSSVFIFPPKPKDVLTITLTPKVTCVVVDISKDDPEVQFSWFVDDVEVHTAQTQPREEQFNSTFRSVSELPIMHQDWLNGKEFKCRVNSAAFPAPIEKTISKTKGRPKAPQVYTIPPPKEQMAKDKVSLTCMITDFFPEDITVEWQWNGQPAENYKNTQPIMDTDGSYFVYSKLNVQKSNWEAGNTFTCSVLHEGLHNHHTEKSLSHSPG

SEQ ID NO: 117 - protein, 106 aa, synthetic construct
  source 1..106: note = Synthetic Polypeptide
GQPKSSPSVTLFPPSSEELETNKATLVCTITDFYPGVVTVDWKVDGTPVTQGMETTQPSKQSNNKYMASSYLTLTARAWERHSSYSCQVTHEGHTVEKSLSRADCS

SEQ ID NO: 118 - protein, 6 aa, synthetic construct
  source 1..6: note = Synthetic Polypeptide
KALDEN